European Patent Specification EP 3 947 675 B1, published August 9, 2023. Title: Method of amplifying mRNAs and for preparing full length mRNA libraries. Applicant: baseclick GmbH. Application TBD. The sequence listing filed with the application follows.

SEQUENCE LISTING (25 sequences)

SEQ ID NO: 1 - DNA, 42 bp, artificial sequence
  Poly(dT) Primer
  misc_feature (41)..(41): v is a, c or g
  misc_feature (42)..(42): n is a, c, g, or t
gtgactggagttcagacgtgttttttttttttttttttttvn

SEQ ID NO: 2 - DNA, 59 bp, artificial sequence
  Alkyne Adapter
  misc_binding (1)..(1): modified with 5'-Hexynyl linker
tagatcggaagagcgtcgtgtagggaaagagtgtagatctcggtggtcgccgtatcatt

SEQ ID NO: 3 - DNA, 19 bp, artificial sequence
  Adapter Primer1
cgacgctcttccgatctac

SEQ ID NO: 4 - DNA, 21 bp, artificial sequence
  Poly(dT) Primer Reverse
gtgactggagttcagacgtgt

SEQ ID NO: 5 - DNA, 18 bp, artificial sequence
  GAPDH Intern Reverse Primer
ggagggatctcgctcctg

SEQ ID NO: 6 - DNA, 20 bp, artificial sequence
  GAPDH Intern Forward Primer
atggggaaggtgaaggtcgg

SEQ ID NO: 7 - DNA, 19 bp, artificial sequence
  eGFP Intern Reverse Primer
gccgtaggtcagggtggtc

SEQ ID NO: 8 - DNA, 21 bp, artificial sequence
  eGFP Intern Forward Primer
gcgaactagtaagcaaggagg

SEQ ID NO: 9 - DNA, 20 bp, artificial sequence
  Cas9 Intern Reverse Primer
ccaccaggaagctctcctcc

SEQ ID NO: 10 - DNA, 20 bp, artificial sequence
  Cas9 Intern Forward Primer
atggcccccaagaagaagcg

SEQ ID NO: 11 - DNA, 18 bp, artificial sequence
  ß-Gal Intern Reverse Primer
gcactccagccagctctc

SEQ ID NO: 12 - DNA, 22 bp, artificial sequence
  ß-Gal Intern Forward Primer
atgagcttcaccctgaccaaca

SEQ ID NO: 13 - DNA, 21 bp, artificial sequence
  FLUC Intern Reverse Primer
gttgtagatgtcgttggcggg

SEQ ID NO: 14 - DNA, 22 bp, artificial sequence
  FLUC Intern Forward Primer
atggaggacgccaagaacatca

SEQ ID NO: 15 - DNA, 58 bp, artificial sequence
  Alkyne Oligo1
  misc_binding (1)..(1): modified with 5'-alkyne dT
aatgatacggcgaccaccgagatctacactctttccctacacgacgctcttccgatct

SEQ ID NO: 16 - RNA, 58 nt, artificial sequence
  Model RNA
uucgacaaacgaaaacacaaacacaaaccaaacagaaaacaguacauguaaucgacca

SEQ ID NO: 17 - DNA, 17 bp, artificial sequence
  Primer1
  misc_binding (1)..(1): modified with FAM
tggtcgattacatgtac

SEQ ID NO: 18 - DNA, 23 bp, artificial sequence
  Primer2
tggtcgattacatgtactgtttt

SEQ ID NO: 19 - DNA, 17 bp, artificial sequence
  Primer3
agatcggaagagcgtcg

SEQ ID NO: 20 - DNA, 57 bp, artificial sequence
  Resulting cDNA after reverse transcription
  misc_binding (1)..(1): modified with FAM
  misc_binding (57)..(57): modified with N3
tggtcgattacatgtactgttttctgtttggtttgtgtttgtgttttcgtttgtcga

SEQ ID NO: 21 - DNA, 116 bp, artificial sequence
  Resulting click product
  misc_binding (1)..(1): modified with FAM
tggtcgattacatgtactgttttctgtttggtttgtgtttgtgttttcgtttgtcgataatgatacggcgaccaccgagatctacactctttccctacacgacgctcttccgatct

SEQ ID NO: 22 - DNA, 116 bp, artificial sequence; identical to SEQ ID NO: 21
  Resulting PCR product

SEQ ID NO: 23 - DNA, 21 bp, artificial sequence
  Oligo2
ttggtatcgctatcgctatgg

SEQ ID NO: 24 - DNA, 32 bp, artificial sequence
  Alkyne-Oligo3
  misc_binding (1)..(1): modified with 5'-Hexynyl linker
aaaaaaaccatgaacaaaatgtgactcatatc

SEQ ID NO: 25 - DNA, 21 bp, artificial sequence
  Azide-Oligo2
  misc_binding (21)..(21): modified with 3'-Azide, 5-methylcytosine
ttggtatcgctatcgctatgg